European Patent Application EP 4 403 581 A1, published July 24, 2024. Title: Anti-CK2alpha antibody or a fragment thereof. Applicant: 公立大学法人福島県立医科大学. Application JP. The sequence listing filed with the application follows.

SEQUENCE LISTING (66 sequences)

SEQ ID NO: 1 - DNA, 1176 bp, Homo sapiens
  source 1..1176: mol_type = other DNA
atgtcgggacccgtgccaagcagggccagagtttacacagatgttaatacacacagacctcgagaatactgggattacgagtcacatgtggtggaatggggaaatcaagatgactaccagctggttcgaaaattaggccgaggtaaatacagtgaagtatttgaagccatcaacatcacaaataatgaaaaagttgttgttaaaattctcaagccagtaaaaaagaagaaaattaagcgtgaaataaagattttggagaatttgagaggaggtcccaacatcatcacactggcagacattgtaaaagaccctgtgtcacgaacccccgccttggtttttgaacacgtaaacaacacagacttcaagcaattgtaccagacgttaacagactatgatattcgattttacatgtatgagattctgaaggccctggattattgtcacagcatgggaattatgcacagagatgtcaagccccataatgtcatgattgatcatgagcacagaaagctacgactaatagactggggtttggctgagttttatcatcctggccaagaatataatgtccgagttgcttcccgatacttcaaaggtcctgagctacttgtagactatcagatgtacgattatagtttggatatgtggagtttgggttgtatgctggcaagtatgatctttcggaaggagccatttttccatggacatgacaattatgatcagttggtgaggatagccaaggttctggggacagaagatttatatgactatattgacaaatacaacattgaattagatccacgtttcaatgatatcttgggcagacactctcgaaagcgatgggaacgctttgtccacagtgaaaatcagcaccttgtcagccctgaggccttggatttcctggacaaactgctgcgatatgaccaccagtcacggcttactgcaagagaggcaatggagcacccctatttctacactgttgtgaaggaccaggctcgaatgggttcatctagcatgccagggggcagtacgcccgtcagcagcgccaatatgatgtcagggatttcttcagtgccaaccccttcaccccttggacctctggcaggctcaccagtgattgctgctgccaacccccttgggatgcctgttccagctgccgctggcgctcagcagtaa

SEQ ID NO: 2 - protein, 391 aa, Homo sapiens
MSGPVPSRARVYTDVNTHRPREYWDYESHVVEWGNQDDYQLVRKLGRGKYSEVFEAINITNNEKVVVKILKPVKKKKIKREIKILENLRGGPNIITLADIVKDPVSRTPALVFEHVNNTDFKQLYQTLTDYDIRFYMYEILKALDYCHSMGIMHRDVKPHNVMIDHEHRKLRLIDWGLAEFYHPGQEYNVRVASRYFKGPELLVDYQMYDYSLDMWSLGCMLASMIFRKEPFFHGHDNYDQLVRIAKVLGTEDLYDYIDKYNIELDPRFNDILGRHSRKRWERFVHSENQHLVSPEALDFLDKLLRYDHQSRLTAREAMEHPYFYTVVKDQARMGSSSMPGGSTPVSSANMMSGISSVPTPSPLGPLAGSPVIAAANPLGMPVPAAAGAQQ

SEQ ID NO: 3 - DNA, 1053 bp, Homo sapiens
  source 1..1053: mol_type = other DNA
atgcccggcccggccgcgggcagcagggcccgggtctacgccgaggtgaacagtctgaggagccgcgagtactgggactacgaggctcacgtcccgagctggggtaatcaagatgattaccaactggttcgaaaacttggtcggggaaaatatagtgaagtatttgaggccattaatatcaccaacaatgagagagtggttgtaaaaatcctgaagccagtgaagaaaaagaagataaaacgagaggttaagattctggagaaccttcgtggtggaacaaatatcattaagctgattgacactgtaaaggaccccgtgtcaaagacaccagctttggtatttgaatatatcaataatacagattttaagcaactctaccagatcctgacagactttgatatccggttttatatgtatgaactacttaaagctctggattactgccacagcaagggaatcatgcacagggatgtgaaacctcacaatgtcatgatagatcaccaacagaaaaagctgcgactgatagattggggtctggcagaattctatcatcctgctcaggagtacaatgttcgtgtagcctcaaggtacttcaagggaccagagctcctcgtggactatcagatgtatgattatagcttggacatgtggagtttgggctgtatgttagcaagcatgatctttcgaagggaaccattcttccatggacaggacaactatgaccagcttgttcgcattgccaaggttctgggtacagaagaactgtatgggtatctgaagaagtatcacatagacctagatccacacttcaacgatatcctgggacaacattcacggaaacgctgggaaaactttatccatagtgagaacagacaccttgtcagccctgaggccctagatcttctggacaaacttctgcgatacgaccatcaacagagactgactgccaaagaggccatggagcacccatacttctaccctgtggtgaaggagcagtcccagccttgtgcagacaatgctgtgctttccagtggtctcacggcagcacgatga

SEQ ID NO: 4 - protein, 350 aa, Homo sapiens
MPGPAAGSRARVYAEVNSLRSREYWDYEAHVPSWGNQDDYQLVRKLGRGKYSEVFEAINITNNERVVVKILKPVKKKKIKREVKILENLRGGTNIIKLIDTVKDPVSKTPALVFEYINNTDFKQLYQILTDFDIRFYMYELLKALDYCHSKGIMHRDVKPHNVMIDHQQKKLRLIDWGLAEFYHPAQEYNVRVASRYFKGPELLVDYQMYDYSLDMWSLGCMLASMIFRREPFFHGQDNYDQLVRIAKVLGTEELYGYLKKYHIDLDPHFNDILGQHSRKRWENFIHSENRHLVSPEALDLLDKLLRYDHQQRLTAKEAMEHPYFYPVVKEQSQPCADNAVLSSGLTAAR

SEQ ID NO: 5 - protein, 5 aa, Mus musculus
DYQMH

SEQ ID NO: 6 - protein, 17 aa, Mus musculus
VIDPGTGGTAYNQKFKG

SEQ ID NO: 7 - skipped

SEQ ID NO: 8 - protein, 11 aa, Mus musculus
RASQDIGSSLN

SEQ ID NO: 9 - protein, 7 aa, Mus musculus
ATSSLDS

SEQ ID NO: 10 - protein, 9 aa, Mus musculus
LQYAIFPYT

SEQ ID NO: 11 - protein, 168 aa, Mus musculus
MEWSWVFLFLLSVIAGVQSQVQLQQSGAELVRPGASVTLSCKASGYKFTDYQMHWVKQTPVHGLEWIGVIDPGTGGTAYNQKFKGKAILTADKSSSTAYMELRSLTSEDSAVYYCTGFVWGTGTTVTVSSAKTTPPSVYPLAPGCGDTTGSSVTLGCLVKGYFPESVT

SEQ ID NO: 12 - protein, 159 aa, Mus musculus
MDMRAPAQIFGFLLLLFPGSRCDIQMTQSPSSLSASLGERVSLTCRASQDIGSSLNWLQQEPDGTIKRLIYATSSLDSGVPKRFSGSRSGSDYSLTISSLESEDFVDYYCLQYAIFPYTFGGGTKLEIKRADAAPTVSIFPPSSEQLTSGGASVVCFLN

SEQ ID NO: 13 - DNA, 498 bp, Mus musculus
  source 1..498: mol_type = other DNA
atggaatggagctgggtctttctcttcctcctgtcagtaattgcaggtgtccaatcccaggttcaactgcagcagtctggggctgagctggtgaggcctggggcttcagtgacgctgtcctgcaaggcttcgggctacaaatttactgactatcaaatgcactgggtgaagcagacacctgttcatggcctggaatggattggagttattgatcctggaactggtggtactgcctacaatcagaagttcaagggcaaggccatactgactgcagacaaatcctccagtacagcctacatggaactccgcagcctgacatctgaagactctgccgtctattactgtacgggatttgtctggggcacagggaccacggtcaccgtctcctcagccaaaacaacacccccatcagtctatccactggcccctgggtgtggagatacaactggttcctctgtgactctgggatgcctggtcaagggctacttccctgagtca

SEQ ID NO: 14 - DNA, 479 bp, Mus musculus
  source 1..479: mol_type = other DNA
atggacatgagggctcctgcacagatttttggcttcttgttgctcttgtttccaggtagcagatgtgacatccagatgacccagtctccatcctccttatctgcctctctgggagaaagagtcagtctcacttgtcgggcaagtcaggacattggtagtagcttaaactggcttcagcaggagccagatggaactattaaacgcctgatctacgccacatccagtttagattctggtgtccccaaaaggttcagtggcagtaggtctgggtcagattattctctcaccatcagcagccttgagtctgaagattttgtagactattactgtctacagtatgctatttttccgtacacgttcggaggggggaccaagctggaaataaaacgggctgatgctgcaccaactgtatccatcttcccaccatccagtgagcagttaacatctggaggtgcctcagtcgtgtgcttcttgaacaa

SEQ ID NO: 15 - protein, 137 aa, Mus musculus
MEWSWVFLFLLSVIAGVQSQVQLQQSGAELVRPGASVTLSCKASGYTFTDYQMHWVKQTPVHGLEWIGVIDPGTGGTAYNQKFKGKAILTADKSSNTAYMELRSLTSEDSAVYYCTGFVWGTGSPVTVSSAKTTPPS

SEQ ID NO: 16 - protein, 135 aa, Mus musculus
MDMRAPAQIFGFLLLLFPGSRCDIQMTQSPSSLSASLGERVSLTCRASQDIGNNLNWLQQEPDGTIKRLIYATSSLDSGVPKRFTGSRSGSDYSLTISSLESEDFVDYYCLQYAIFPYTFGGGTKLEIKRADAAP

SEQ ID NO: 17 - protein, 5 aa, Mus musculus
DYQMH

SEQ ID NO: 18 - protein, 17 aa, Mus musculus
VIDPGTGGTAYNQKFKG

SEQ ID NO: 19 - skipped

SEQ ID NO: 20 - protein, 11 aa, Mus musculus
RASQDIGNNLN

SEQ ID NO: 21 - protein, 7 aa, Mus musculus
ATSSLDS

SEQ ID NO: 22 - protein, 9 aa, Mus musculus
LQYAIFPYT

SEQ ID NO: 23 - protein, 137 aa, Mus musculus
MEWSWVFLFLLSVIAGVQSQVQLQQSGAELVRPGASVTLSCKASGYTFTDFQMHWVKQTPVHGLEWIGVIDPGTGGTAYNQKFKDKAILTADKSSNTAYMELRSLTSEDSAVYYCTGFVWGTGTTVTVSSAKTTPPS

SEQ ID NO: 24 - protein, 135 aa, Mus musculus; identical to SEQ ID NO: 16

SEQ ID NO: 25 - protein, 5 aa, Mus musculus
DFQMH

SEQ ID NO: 26 - protein, 17 aa, Mus musculus
VIDPGTGGTAYNQKFKD

SEQ ID NO: 27 - skipped

SEQ ID NO: 28 - protein, 11 aa, Mus musculus
RASQDIGNNLN

SEQ ID NO: 29 - protein, 7 aa, Mus musculus
ATSSLDS

SEQ ID NO: 30 - protein, 9 aa, Mus musculus
LQYAIFPYT

SEQ ID NO: 31 - protein, 137 aa, Mus musculus
MEWSWVFLFLLSVIAGVQSQVQLQQSGAELVRPGASVTLSCKASGYKFTDYQMHWVKQTPVHGLEWIGVLDPGTGGTAYNQKFRGKAILTADKSSSTAYMELRSLTSEDSAVYYCTGFVWGTGTTVTVSSAKTTPPS

SEQ ID NO: 32 - protein, 135 aa, Mus musculus
MDMRAPAQIFGFLLLLFPGSRCDIQMTQSPSSLSASLGERVSLTCRASQDIGSSLNWLQQEPDGTIKRLIYATSSLDSGVPKRFSGSRSGSDYSLTISSLESEDFVDYYCLQYAIFPYTFGGGTKLEIKRADAAP

SEQ ID NO: 33 - protein, 5 aa, Mus musculus
DYQMH

SEQ ID NO: 34 - protein, 17 aa, Mus musculus
VLDPGTGGTAYNQKFRG

SEQ ID NO: 35 - skipped

SEQ ID NO: 36 - protein, 11 aa, Mus musculus
RASQDIGSSLN

SEQ ID NO: 37 - protein, 7 aa, Mus musculus
ATSSLDS

SEQ ID NO: 38 - protein, 9 aa, Mus musculus
LQYAIFPYT

SEQ ID NO: 39 - protein, 188 aa, Mus musculus
MSSPQTLNTLTLTMGWSWIFLFLLSGTAGVHSEVQLQQSGPVLVKPGASVKMSCKASGYTFTDYYMNWVKQSHGKSLEWIGVIDPNNGGTSYNQKFKGKATLTVDKSSSTAYMELNSLTSEDSAVYYCPRMGGNFYFDYWGQGTTLTVSSAKTTPPSVYPLAPGSAAQTNSMVTLGCLVKGYFPEPVT

SEQ ID NO: 40 - protein, 162 aa, Mus musculus
MRCLAEFLGLLVLWIPGAIGDIVMTQAAPSVPVTPGESVSISCRSSKSLLHSNGNTYLYWFLQRPGQSPQLLIYRMSNLASGVPDRFSGSGSGTAFTLRISRVEAEDVGVYYCMQHLEFPYTFGGGTKLEIKRADAAPTVSIFPPSSEQLTSGGASVVCFLN

SEQ ID NO: 41 - protein, 5 aa, Mus musculus
DYYMN

SEQ ID NO: 42 - protein, 17 aa, Mus musculus
VIDPNNGGTSYNQKFKG

SEQ ID NO: 43 - protein, 9 aa, Mus musculus
MGGNFYFDY

SEQ ID NO: 44 - protein, 16 aa, Mus musculus
RSSKSLLHSNGNTYLY

SEQ ID NO: 45 - protein, 7 aa, Mus musculus
RMSNLAS

SEQ ID NO: 46 - protein, 9 aa, Mus musculus
MQHLEFPYT

SEQ ID NO: 47 - protein, 185 aa, Mus musculus
MSSSQSLNTLTLTMEWIWIFLFILSGTAGVQSQVQLQQSGAELTRPGASVKLSCKASGYTFTSFGISWVKQTTGQGLEWIGEIYPRSGNTYYNEKFKGKATLTADKSSSTAFMELRSLTTEDSAVYFCEGDWYFDVWGTGTTVTVSSAKTTPPSVYPLAPGSAAQTNSMVTLGCLVKGYFPEPVT

SEQ ID NO: 48 - protein, 162 aa, Mus musculus
MMSPAQFLFLSVLWIRETNGDVVMTQTPLTLSVTIGQPASISCKSSQSLLDSDGKTYLNWLLQRPGQSPKRLIYLVSKLDSGVPDRFTGSGSGTDFTLKISRVEAEDLGVYYCWQGTHFPHTFGGGTKLEMKRADAAPTVSIFPPSSEQLTSGGASVVCFLN

SEQ ID NO: 49 - protein, 5 aa, Mus musculus
SFGIS

SEQ ID NO: 50 - protein, 17 aa, Mus musculus
EIYPRSGNTYYNEKFKG

SEQ ID NO: 51 - protein, 6 aa, Mus musculus
DWYFDV

SEQ ID NO: 52 - protein, 16 aa, Mus musculus
KSSQSLLDSDGKTYLN

SEQ ID NO: 53 - protein, 7 aa, Mus musculus
LVSKLDS

SEQ ID NO: 54 - protein, 9 aa, Mus musculus
WQGTHFPHT

SEQ ID NO: 55 - DNA, 431 bp, Mus musculus
  source 1..431: mol_type = other DNA
aagacactgactctaaccatggaatggagctgggtctttctcttcctcctgtcagtaattgcaggtgtccaatcccaggttcaactgcagcagtctggggctgagctggtgaggcctggggcttcagtgacgctgtcctgcaaggcttcgggctacacatttactgactatcaaatgcactgggtgaagcagacacctgttcatggcctggaatggattggagttattgatcctggaactggtggtactgcctacaatcagaagttcaagggcaaggccatactgactgcagacaaatcctccaacacagcctacatggagctccgcagcctgacatctgaagactctgccgtctattactgtacgggatttgtctggggcacagggtccccggtcaccgtctcctcagccaaaacaacacccccatcagt

SEQ ID NO: 56 - DNA, 425 bp, Mus musculus
  source 1..425: mol_type = other DNA
attgcagtcaggactcagcatggacatgagggctcctgcacagatttttggcttcttgttgctcttgtttccaggtagcagatgtgacatccagatgacccagtctccgtcctccttatctgcctctctgggagaaagagtcagtctcacttgtcgggcaagtcaggacattggtaataacttaaactggcttcagcaggagccagatggaactattaaacgcctgatctacgccacatccagtttagattctggtgtccccaaaaggttcactggcagtaggtctgggtcagattattctctcaccatcagcagccttgagtctgaagattttgttgactattactgtctacaatatgctatttttccgtacacgttcggaggggggaccaagctggaaataaaacgggctgatgctgcaccaa

SEQ ID NO: 57 - DNA, 422 bp, Mus musculus
  source 1..422: mol_type = other DNA
actctaaccatggaatggagctgggtctttctcttcctcctgtcagtaattgcaggtgtccaatcccaggttcaactgcagcagtctggggctgagctggtgaggcctggggcttcagtgacgctgtcctgcaaggcttcgggctacacatttactgactttcaaatgcactgggtgaagcagacacctgttcatggcctggaatggattggagttattgatcctggaactggtggtactgcctacaatcagaagttcaaggacaaggccatactgactgcagacaaatcctccaacacagcctacatggagctccgcagcctgacatctgaggactctgccgtctattactgtacggggtttgtctggggcacagggaccacggtcaccgtctcctcagccaaaacaacacccccatcagt

SEQ ID NO: 58 - DNA, 413 bp, Mus musculus
  source 1..413: mol_type = other DNA
actcagcatggacatgagggctcctgcacagatttttggcttcttgttgctcttgtttccaggtagcagatgtgacatccagatgacccagtctccgtcctccttatctgcctctctgggagaaagagtcagtctcacttgtcgggcaagtcaggacattggtaataacttaaactggcttcagcaggagccagatggaactattaaacgcctgatctacgccacatccagtttagattctggtgtccccaaaaggttcactggcagtaggtctgggtcagattattctctcaccatcagcagccttgagtctgaagattttgtagactattactgtctacagtatgctatttttccgtacacgttcggaggggggaccaagctggaaataaaacgggctgatgctgcaccaa

SEQ ID NO: 59 - DNA, 426 bp, Mus musculus
  source 1..426: mol_type = other DNA
actgactctaaccatggaatggagctgggtctttctcttcctcctgtcagtaattgcaggtgtccaatcccaggttcaactgcagcagtctggggctgagctggtgaggcctggggcttcagtgacgctgtcctgcaaggcttcgggctacaaatttactgactatcaaatgcactgggtgaagcagacacctgttcatggcctggaatggattggagttcttgatcctggaactggtggtactgcctacaatcagaagttcaggggcaaggccatactgactgcagacaaatcctccagtacagcctacatggaactccgcagcctgacatctgaagactctgccgtctattattgtacgggatttgtctggggcacagggaccacggtcaccgtctcctcagccaaaacaacacccccatcagt

SEQ ID NO: 60 - DNA, 417 bp, Mus musculus
  source 1..417: mol_type = other DNA
caggactcagcatggacatgagggctcctgcacagatttttggcttcttgttgctcttgtttccaggtagcagatgtgacatccagatgacccagtctccatcctccttatctgcctctctgggagaaagagtcagtctcacttgtcgggcaagtcaggacattggtagtagcttaaactggcttcagcaggagccagatggaactattaaacgcctgatctacgccacatccagtttagattctggtgtccccaaaaggttcagtggcagtaggtctgggtcagattattctctcaccatcagcagccttgagtctgaagattttgtggactattactgtctacagtatgctatttttccgtacacgttcggaggggggaccaagctggaaataaaacgggctgatgctgcaccaa

SEQ ID NO: 61 - DNA, 575 bp, Mus musculus
  source 1..575: mol_type = other DNA
acatgtccaatgtcctctccacagacactgaacacactgactctaaccatgggatggagctggatctttctcttcctcctgtcaggaactgcaggtgtccactctgaggtccagctgcaacagtctggacctgtgctggtgaagcctggggcttcagtgaagatgtcctgtaaggcttctggatacacattcactgactactatatgaactgggtgaagcagagccatggaaagagccttgagtggattggagttattgatcctaacaacggtggtactagctacaaccagaagttcaagggcaaggccacattgactgttgacaagtcctccagcacagcctacatggagctcaacagcctgacatctgaggactctgcagtctattactgtccaagaatggggggtaacttttactttgactactggggccaaggcaccactctcacagtctcctcagccaaaacgacacccccatctgtctatccactggcccctggatctgctgcccaaactaactccatggtgaccctgggatgcctggtcaagggctatttccctgagccagtgacagt

SEQ ID NO: 62 - DNA, 516 bp, Mus musculus
  source 1..516: mol_type = other DNA
atcactctcctatgttcatttcctcaaaatgatgagtcctgcccagttcctgtttctgtcagtgctctggattcgggaaaccaacggtgatgttgtgatgacccagactccactcactttgtcggttaccattggacaaccagcctccatctcttgcaagtcaagtcagagcctcttagatagtgatggaaagacatatttgaattggttgttacagaggccaggccagtctccaaagcgcctaatctatctggtgtctaaactggactctggagtccctgacaggttcactggcagtggatcagggacagatttcacactgaaaatcagcagagtggaggctgaggatttgggagtttattattgctggcaaggtacacattttcctcacacgttcggaggggggaccaagctggaaatgaaacgggctgatgctgcaccaactgtatccatcttcccaccatccagtgagcagttaacatctggaggtgcctcagtcgtgtgcttcttgaacaa

SEQ ID NO: 63 - DNA, 546 bp, Mus musculus
  source 1..546: mol_type = other DNA
acagtccctgaacacactgactctaaccatggaatggatctggatctttctcttcatcctgtcaggaactgcaggtgtccaatcccaggttcagctgcagcagtctggagctgagctgacgaggcctggggcttcagtgaagctgtcctgcaaggcttctggctacaccttcacaagctttggtataagctgggtgaagcagacaactggacagggccttgagtggattggagagatttatcctagaagtggtaatacttactacaatgagaaattcaagggcaaggccacactgactgcagacaaatcctccagcacagcgttcatggagctccgcagcctgacaactgaggactctgcggtctatttctgtgagggagactggtacttcgatgtctggggcacagggaccacggtcaccgtctcctcagccaaaacgacacccccatctgtctatccactggcccctggatctgctgcccaaactaactccatggtgaccctgggatgcctggtcaagggctatttccctgagccagtgacagt

SEQ ID NO: 64 - DNA, 505 bp, Mus musculus
  source 1..505: mol_type = other DNA
atcactctcctatgttcatttcctcaaaatgatgagtcctgcccagttcctgtttctgtcagtgctctggattcgggaaaccaacggtgatgttgtgatgacccagactccactcactttgtcggttaccattggacaaccagcctccatctcttgcaagtcaagtcagagcctcttagatagtgatggaaagacatatttgaattggttgttacagaggccaggccagtctccaaagcgcctaatctatctggtgtctaaactggactctggagtccctgacaggttcactggcagtggatcagggacagatttcacactgaaaatcagcagagtggaggctgaggatttgggagtttattattgctggcaaggtacacattttcctcacacgttcggaggggggaccaagctggaaatgaaacgggctgatgctgcaccaactgtatccatcttcccaccatccagtgagcagttaacatctggaggtgcctcagtcgtgtgc

SEQ ID NO: 65 - DNA, 21 bp, synthetic construct
  source 1..21: mol_type = other DNA
gaggctaacgattggtcagtg

SEQ ID NO: 66 - DNA, 20 bp, synthetic construct
  source 1..20: mol_type = other DNA
ttctaacgggtctgggagtt